European Patent Specification EP 3 523 659 B1, published August 14, 2024. Title: Multi-protease method. Applicant: Oblique Therapeutics AB. The sequence listing filed with the application follows.

SEQUENCE LISTING (184 sequences)

SEQ ID NO: 1 - protein, 839 aa, Homo sapiens [sequence omitted]

SEQ ID NO: 2 - protein, 13 aa, Artificial Sequence
  peptide sequence
LLSQDSVAASTEK

SEQ ID NO: 3 - protein, 16 aa, Artificial Sequence
  peptide sequence
LLSQDSVAASTEKTLR

SEQ ID NO: 4 - protein, 23 aa, Artificial Sequence
  peptide sequence
QFSGSLKPEDAEVFKSPAASGEK

SEQ ID NO: 5 - protein, 22 aa, Artificial Sequence
  peptide sequence
LLSQDSVAASTEKTLRLYDRRS

SEQ ID NO: 6 - protein, 15 aa, Artificial Sequence
  peptide sequence
GRHWKNFALVPLLRE

SEQ ID NO: 7 - protein, 16 aa, Artificial Sequence
  peptide sequence
LVENGADVQAAAHGDF

SEQ ID NO: 8 - protein, 11 aa, Artificial Sequence
  peptide sequence
DGPTGARLLSQ

SEQ ID NO: 9 - protein, 14 aa, Artificial Sequence
  peptide sequence
DAEVFKSPAASGEK

SEQ ID NO: 10 - protein, 13 aa, Artificial Sequence
  peptide sequence
SQDSVAASTEKTL

SEQ ID NO: 11 - protein, 12 aa, Artificial Sequence
  peptide sequence
SGSLKPEDAEVF

SEQ ID NO: 12 - protein, 12 aa, Artificial Sequence
  peptide sequence
VSPVITIQRPGD

SEQ ID NO: 13 - protein, 17 aa, Artificial Sequence
  peptide sequence
VSPVITIQRPGDGPTGA

SEQ ID NO: 14 - protein, 15 aa, Artificial Sequence
  peptide sequence
LNLHDGQNTTIPLLL

SEQ ID NO: 15 - protein, 9 aa, Artificial Sequence
  peptide sequence
YTDSYYKGQ

SEQ ID NO: 16 - protein, 9 aa, Artificial Sequence
  peptide sequence
SLPSESTSH

SEQ ID NO: 17 - protein, 11 aa, Artificial Sequence
  peptide sequence
EDPGNCEGVKR

SEQ ID NO: 18 - protein, 13 aa, Artificial Sequence
  peptide sequence
DRQSAQPEEVYLR

SEQ ID NO: 19 - protein, 11 aa, Artificial Sequence
  peptide sequence
QSAQPEEVYLR

SEQ ID NO: 20 - protein, 16 aa, Artificial Sequence
  peptide sequence
FAPQIRVNLNYRKGTG

SEQ ID NO: 21 - protein, 13 aa, Artificial Sequence
  peptide sequence
ASQPDPNRFDRDR

SEQ ID NO: 22 - protein, 15 aa, Artificial Sequence
  peptide sequence
LNLKDGVNACILPLL

SEQ ID NO: 23 - protein, 9 aa, Artificial Sequence
  peptide sequence
CTDDYYRGH

SEQ ID NO: 24 - protein, 16 aa, Artificial Sequence
  peptide sequence
LVENGANVHARACGRF

SEQ ID NO: 25 - protein, 10 aa, Artificial Sequence
  peptide sequence
EDPSGAGVPR

SEQ ID NO: 26 - protein, 15 aa, Artificial Sequence
  peptide sequence
GASEENYVPVQLLQS

SEQ ID NO: 27 - protein, 15 aa, Artificial Sequence
  peptide sequence
WSSTDLGAAADPLQK

SEQ ID NO: 28 - protein, 13 aa, Artificial Sequence
  peptide sequence
LLSQDSVAASTEK

SEQ ID NO: 29 - protein, 16 aa, Artificial Sequence
  peptide sequence
LLSQDSVAASTEKTLR

SEQ ID NO: 30 - protein, 21 aa, Artificial Sequence
  peptide sequence
AMLNLHDGQNTTIPLLLEIAR

SEQ ID NO: 31 - protein, 19 aa, Artificial Sequence
  peptide sequence
QTDSLKELVNASYTDSYYK

SEQ ID NO: 32 - protein, 11 aa, Artificial Sequence
  peptide sequence
GQTALHIAIER

SEQ ID NO: 33 - protein, 26 aa, Artificial Sequence
  peptide sequence
NMALVTLLVENGADVQAAAHGDFFKK

SEQ ID NO: 34 - protein, 15 aa, Artificial Sequence
  peptide sequence
FLLQNSWQTADISAR

SEQ ID NO: 35 - protein, 23 aa, Artificial Sequence
  peptide sequence
DSVGNTVLHALVEVADNTADNTK

SEQ ID NO: 36 - protein, 13 aa, Artificial Sequence
  peptide sequence
LHPTLKLEELTNK

SEQ ID NO: 37 - protein, 14 aa, Artificial Sequence
  peptide sequence
KGMTPLALAAGTGK

SEQ ID NO: 38 - protein, 13 aa, Artificial Sequence
  peptide sequence
GMTPLALAAGTGK

SEQ ID NO: 39 - protein, 10 aa, Artificial Sequence
  peptide sequence
IGVLAYILQR

SEQ ID NO: 40 - protein, 9 aa, Artificial Sequence
  peptide sequence
AITILDTEK

SEQ ID NO: 41 - protein, 7 aa, Artificial Sequence
  peptide sequence
TLSFSLR

SEQ ID NO: 42 - protein, 9 aa, Artificial Sequence
  peptide sequence
NFALVPLLR

SEQ ID NO: 43 - protein, 18 aa, Artificial Sequence
  peptide sequence
EASARDRQSAQPEEVYLR

SEQ ID NO: 44 - protein, 13 aa, Artificial Sequence
  peptide sequence
DRQSAQPEEVYLR

SEQ ID NO: 45 - protein, 11 aa, Artificial Sequence
  peptide sequence
QSAQPEEVYLR

SEQ ID NO: 46 - protein, 15 aa, Artificial Sequence
  peptide sequence
QFSGSLKPEDAEVFK

SEQ ID NO: 47 - protein, 23 aa, Artificial Sequence
  peptide sequence
QFSGSLKPEDAEVFKSPAASGEK

SEQ ID NO: 48 - protein, 11 aa, Artificial Sequence
  peptide sequence
DGPTGARLLSQ

SEQ ID NO: 49 - protein, 14 aa, Artificial Sequence
  peptide sequence
DSVAASTEKTLRLY

SEQ ID NO: 50 - protein, 17 aa, Artificial Sequence
  peptide sequence
DGQNTTIPLLLEIARQT

SEQ ID NO: 51 - protein, 12 aa, Artificial Sequence
  peptide sequence
DSLKELVNASYT

SEQ ID NO: 52 - protein, 15 aa, Artificial Sequence
  peptide sequence
DSVGNTVLHALVEVA

SEQ ID NO: 53 - protein, 14 aa, Artificial Sequence
  peptide sequence
DAEVFKSPAASGEK

SEQ ID NO: 54 - protein, 14 aa, Artificial Sequence
  peptide sequence
LSQDSVAASTEKTL

SEQ ID NO: 55 - protein, 13 aa, Artificial Sequence
  peptide sequence
SQDSVAASTEKTL

SEQ ID NO: 56 - protein, 16 aa, Artificial Sequence
  peptide sequence
SQDSVAASTEKTLRLY

SEQ ID NO: 57 - protein, 12 aa, Artificial Sequence
  peptide sequence
NLHDGQNTTIPL

SEQ ID NO: 58 - protein, 17 aa, Artificial Sequence
  peptide sequence
LVENGADVQAAAHGDFF

SEQ ID NO: 59 - protein, 16 aa, Artificial Sequence
  peptide sequence
QTADISARDSVGNTVL

SEQ ID NO: 60 - protein, 16 aa, Artificial Sequence
  peptide sequence
HALVEVADNTADNTKF

SEQ ID NO: 61 - protein, 12 aa, Artificial Sequence
  peptide sequence
AAGTGKIGVLAY

SEQ ID NO: 62 - protein, 12 aa, Artificial Sequence
  peptide sequence
SGSLKPEDAEVF

SEQ ID NO: 63 - protein, 10 aa, Artificial Sequence
  peptide sequence
FGKGDSEEAF

SEQ ID NO: 64 - protein, 11 aa, Artificial Sequence
  peptide sequence
HDGQNTTIPLL

SEQ ID NO: 65 - protein, 16 aa, Artificial Sequence
  peptide sequence
LVENGADVQAAAHGDF

SEQ ID NO: 66 - protein, 15 aa, Artificial Sequence
  peptide sequence
VENGADVQAAAHGDF

SEQ ID NO: 67 - protein, 15 aa, Artificial Sequence
  peptide sequence
VENGADVQAAAHGDF

SEQ ID NO: 68 - protein, 16 aa, Artificial Sequence
  peptide sequence
HALVEVADNTADNTKF

SEQ ID NO: 69 - protein, 13 aa, Artificial Sequence
  peptide sequence
VEVADNTADNTKF

SEQ ID NO: 70 - protein, 17 aa, Artificial Sequence
  peptide sequence
EVIAYSSSETPNRHDML

SEQ ID NO: 71 - protein, 17 aa, Artificial Sequence
  peptide sequence
VSPVITIQRPGDGPTGA

SEQ ID NO: 72 - protein, 12 aa, Artificial Sequence
  peptide sequence
IQRPGDGPTGAR

SEQ ID NO: 73 - protein, 12 aa, Artificial Sequence
  peptide sequence
RPGDGPTGARLL

SEQ ID NO: 74 - protein, 15 aa, Artificial Sequence
  peptide sequence
LNLHDGQNTTIPLLL

SEQ ID NO: 75 - protein, 8 aa, Artificial Sequence
  peptide sequence
DTEKSFLK

SEQ ID NO: 76 - protein, 11 aa, Artificial Sequence
  peptide sequence
EDPGNCEGVKR

SEQ ID NO: 77 - protein, 12 aa, Artificial Sequence
  peptide sequence
EDPGNCEGVKRT

SEQ ID NO: 78 - protein, 13 aa, Artificial Sequence
  peptide sequence
EDPGNCEGVKRTL

SEQ ID NO: 79 - protein, 16 aa, Artificial Sequence
  peptide sequence
SARDRQSAQPEEVYLR

SEQ ID NO: 80 - protein, 13 aa, Artificial Sequence
  peptide sequence
DRQSAQPEEVYLR

SEQ ID NO: 81 - protein, 11 aa, Artificial Sequence
  peptide sequence
QSAQPEEVYLR

SEQ ID NO: 82 - protein, 18 aa, Artificial Sequence
  peptide sequence
SSPAGGVLGGGLGGGGGR

SEQ ID NO: 83 - protein, 11 aa, Artificial Sequence
  peptide sequence
FDGGVEAIATR

SEQ ID NO: 84 - protein, 14 aa, Artificial Sequence
  peptide sequence
EKDILTAIAADLCK

SEQ ID NO: 85 - protein, 14 aa, Artificial Sequence
  peptide sequence
FDHIFYTGNTAVGK

SEQ ID NO: 86 - protein, 9 aa, Artificial Sequence
  peptide sequence
ILSLLEGQK

SEQ ID NO: 87 - protein, 12 aa, Artificial Sequence
  peptide sequence
IAFGGETDEATR

SEQ ID NO: 88 - protein, 13 aa, Artificial Sequence
  peptide sequence
IAFGGETDEATRY

SEQ ID NO: 89 - protein, 13 aa, Artificial Sequence
  peptide sequence
YIAPTVLTDVDPK

SEQ ID NO: 90 - protein, 12 aa, Artificial Sequence
  peptide sequence
IAPTVLTDVDPK

SEQ ID NO: 91 - protein, 17 aa, Artificial Sequence
  peptide sequence
VMQEEIFGPILPIVPVK

SEQ ID NO: 92 - protein, 12 aa, Artificial Sequence
  peptide sequence
NVDEAINFINER

SEQ ID NO: 93 - protein, 20 aa, Artificial Sequence
  peptide sequence
QFYDQALQQAVVDDDANNAK

SEQ ID NO: 94 - protein, 14 aa, Artificial Sequence
  peptide sequence
TFHETLDCCGSSTL

SEQ ID NO: 95 - protein, 7 aa, Artificial Sequence
  peptide sequence
IVLSYVR

SEQ ID NO: 96 - protein, 24 aa, Artificial Sequence
  peptide sequence
GISGEKDVSPDLSCADEISECYHK

SEQ ID NO: 97 - protein, 8 aa, Artificial Sequence
  peptide sequence
ETLLEIQK

SEQ ID NO: 98 - protein, 11 aa, Artificial Sequence
  peptide sequence
GQMGPTEQGPY

SEQ ID NO: 99 - protein, 8 aa, Artificial Sequence
  peptide sequence
LCLLPLVR

SEQ ID NO: 100 - protein, 11 aa, Artificial Sequence
  peptide sequence
AWDDFFPGSDR

SEQ ID NO: 101 - protein, 19 aa, Artificial Sequence
  peptide sequence
TPMGIVLDALEQQEEGINR

SEQ ID NO: 102 - protein, 12 aa, Artificial Sequence
  peptide sequence
DALEQQEEGINR

SEQ ID NO: 103 - protein, 7 aa, Artificial Sequence
  peptide sequence
LTDYISK

SEQ ID NO: 104 - protein, 11 aa, Artificial Sequence
  peptide sequence
TVLWGLGVLIR

SEQ ID NO: 105 - protein, 12 aa, Artificial Sequence
  peptide sequence
EADEDAVQFANR

SEQ ID NO: 106 - protein, 15 aa, Artificial Sequence
  peptide sequence
QGGLVDLLWDGGLKR

SEQ ID NO: 107 - protein, 10 aa, Artificial Sequence
  peptide sequence
VIDNGSGMCK

SEQ ID NO: 108 - protein, 10 aa, Artificial Sequence
  peptide sequence
AGFAGDDAPR

SEQ ID NO: 109 - protein, 9 aa, Artificial Sequence
  peptide sequence
AVFPSIVGR

SEQ ID NO: 110 - protein, 8 aa, Artificial Sequence
  peptide sequence
PSIVGRPR

SEQ ID NO: 111 - protein, 11 aa, Artificial Sequence
  peptide sequence
IWHHTFYNELR

SEQ ID NO: 112 - protein, 14 aa, Artificial Sequence
  peptide sequence
TTGIVMDSGDGVTH

SEQ ID NO: 113 - protein, 16 aa, Artificial Sequence
  peptide sequence
SYELPDGQVITIGNER

SEQ ID NO: 114 - protein, 14 aa, Artificial Sequence
  peptide sequence
ELPDGQVITIGNER

SEQ ID NO: 115 - protein, 16 aa, Artificial Sequence
  peptide sequence
ISKQEYDESGPSIVHR

SEQ ID NO: 116 - protein, 12 aa, Artificial Sequence
  peptide sequence
QEYDESGPSIVH

SEQ ID NO: 117 - protein, 13 aa, Artificial Sequence
  peptide sequence
QEYDESGPSIVHR

SEQ ID NO: 118 - protein, 13 aa, Artificial Sequence
  peptide sequence
STPAITLESPDIK

SEQ ID NO: 119 - protein, 17 aa, Artificial Sequence
  peptide sequence
STPAITLESPDIKYPLR

SEQ ID NO: 120 - protein, 12 aa, Artificial Sequence
  peptide sequence
LIDREIISHDTR

SEQ ID NO: 121 - protein, 10 aa, Artificial Sequence
  peptide sequence
IDGNLVVRPY

SEQ ID NO: 122 - protein, 17 aa, Artificial Sequence
  peptide sequence
TPISSDDDKGFVDLVIK

SEQ ID NO: 123 - protein, 9 aa, Artificial Sequence
  peptide sequence
VYFKDTHPK

SEQ ID NO: 124 - protein, 11 aa, Artificial Sequence
  peptide sequence
GPSGLLVYQGK

SEQ ID NO: 125 - protein, 19 aa, Artificial Sequence
  peptide sequence
SVGMIAGGTGITPMLQVIR

SEQ ID NO: 126 - protein, 11 aa, Artificial Sequence
  peptide sequence
DILLRPELEEL

SEQ ID NO: 127 - protein, 9 aa, Artificial Sequence
  peptide sequence
FKLWYTLDR

SEQ ID NO: 128 - protein, 7 aa, Artificial Sequence
  peptide sequence
LWYTLDR

SEQ ID NO: 129 - protein, 18 aa, Artificial Sequence
  peptide sequence
APEAWDYGQGFVNEEMIR

SEQ ID NO: 130 - protein, 7 aa, Artificial Sequence
  peptide sequence
FMLNEVK

SEQ ID NO: 131 - protein, 9 aa, Artificial Sequence
  peptide sequence
TCLLIVFSK

SEQ ID NO: 132 - protein, 10 aa, Artificial Sequence
  peptide sequence
DTAGQEDYDR

SEQ ID NO: 133 - protein, 14 aa, Artificial Sequence
  peptide sequence
HFCPNVPIILVGNK

SEQ ID NO: 134 - protein, 15 aa, Artificial Sequence
  peptide sequence
HFCPNVPIILVGNKK

SEQ ID NO: 135 - protein, 9 aa, Artificial Sequence
  peptide sequence
VPIILVGNK

SEQ ID NO: 136 - protein, 8 aa, Artificial Sequence
  peptide sequence
EVFEMATR

SEQ ID NO: 137 - protein, 16 aa, Artificial Sequence
  peptide sequence
GDSTVNTEPATSSAPR

SEQ ID NO: 138 - protein, 12 aa, Artificial Sequence
  peptide sequence
TASISETPVDVR

SEQ ID NO: 139 - protein, 12 aa, Artificial Sequence
  peptide sequence
SDEEEPKDESAR

SEQ ID NO: 140 - protein, 8 aa, Artificial Sequence
  peptide sequence
EPLEAEAR

SEQ ID NO: 141 - protein, 7 aa, Artificial Sequence
  peptide sequence
ESATPLR

SEQ ID NO: 142 - protein, 18 aa, Artificial Sequence
  peptide sequence
GADDAMESSKPGPVQVVL

SEQ ID NO: 143 - protein, 18 aa, Artificial Sequence
  peptide sequence
ARAAPDPPPLFDDTSGGY

SEQ ID NO: 144 - protein, 16 aa, Artificial Sequence
  peptide sequence
AAPDPPPLFDDTSGGY

SEQ ID NO: 145 - protein, 11 aa, Artificial Sequence
  peptide sequence
LSELDDRADAL

SEQ ID NO: 146 - protein, 18 aa, Artificial Sequence
  peptide sequence
LSELDDRADALQAGASQF

SEQ ID NO: 147 - protein, 17 aa, Artificial Sequence
  peptide sequence
AQLKSEAAGSPDQGSTY

SEQ ID NO: 148 - protein, 22 aa, Artificial Sequence
  peptide sequence
QAQLTQAQAEQPAQSSTEMEEF

SEQ ID NO: 149 - protein, 16 aa, Artificial Sequence
  peptide sequence
SSSAEESGQDVLENTF

SEQ ID NO: 150 - protein, 12 aa, Artificial Sequence
  peptide sequence
NIDVAPGAPQEK

SEQ ID NO: 151 - protein, 18 aa, Artificial Sequence
  peptide sequence
GADDAMESSKPGPVQVVL

SEQ ID NO: 152 - protein, 11 aa, Artificial Sequence
  peptide sequence
SVNAITADGSR

SEQ ID NO: 153 - protein, 7 aa, Artificial Sequence
  peptide sequence
VFLNAKK

SEQ ID NO: 154 - protein, 13 aa, Artificial Sequence
  peptide sequence
AYPSNITSETGFR

SEQ ID NO: 155 - protein, 17 aa, Artificial Sequence
  peptide sequence
TATPPAPDSPQEPLVLR

SEQ ID NO: 156 - protein, 16 aa, Artificial Sequence
  peptide sequence
IMSSNSASAANGNDSK

SEQ ID NO: 157 - protein, 17 aa, Artificial Sequence
  peptide sequence
IMSSNSASAANGNDSKK

SEQ ID NO: 158 - protein, 8 aa, Artificial Sequence
  peptide sequence
TSVTPVLR

SEQ ID NO: 159 - protein, 16 aa, Artificial Sequence
  peptide sequence
AQAALQAVNSVQSGNL

SEQ ID NO: 160 - protein, 13 aa, Artificial Sequence
  peptide sequence
QAVNSVQSGNLAL

SEQ ID NO: 161 - protein, 7 aa, Artificial Sequence
  peptide sequence
TSLNVKY

SEQ ID NO: 162 - protein, 14 aa, Artificial Sequence
  peptide sequence
GLSVPNVHGALAPL

SEQ ID NO: 163 - protein, 14 aa, Artificial Sequence
  peptide sequence
AIPSAAAAAAAAGR

SEQ ID NO: 164 - protein, 12 aa, Artificial Sequence
  peptide sequence
PSAAAAAAAAGR

SEQ ID NO: 165 - protein, 12 aa, Artificial Sequence
  peptide sequence
EGQEDQGLTKDY

SEQ ID NO: 166 - protein, 10 aa, Artificial Sequence
  peptide sequence
QFPGFPAAAY

SEQ ID NO: 167 - protein, 12 aa, Artificial Sequence
  peptide sequence
GPVAAAAVAAAR

SEQ ID NO: 168 - protein, 16 aa, Artificial Sequence
  peptide sequence
SLDPTNAENTASQSPR

SEQ ID NO: 169 - protein, 12 aa, Artificial Sequence
  peptide sequence
KTNEAQAIETAR

SEQ ID NO: 170 - protein, 17 aa, Artificial Sequence
  peptide sequence
SAPNPDDPLANDVAEQW

SEQ ID NO: 171 - protein, 12 aa, Artificial Sequence
  peptide sequence
KTNEAQAIETAR

SEQ ID NO: 172 - protein, 10 aa, Artificial Sequence
  peptide sequence
VYSKDQLQTF

SEQ ID NO: 173 - protein, 14 aa, Artificial Sequence
  peptide sequence
YLPDGSTIEIGPSR

SEQ ID NO: 174 - protein, 13 aa, Artificial Sequence
  peptide sequence
LPDGSTIEIGPSR

SEQ ID NO: 175 - protein, 13 aa, Artificial Sequence
  peptide sequence
SLATQDSDNPDLR

SEQ ID NO: 176 - protein, 19 aa, Artificial Sequence
  peptide sequence
SNLGSTETLEEMPSGSQDK

SEQ ID NO: 177 - protein, 13 aa, Artificial Sequence
  peptide sequence
LNQPVPELSHASL

SEQ ID NO: 178 - protein, 18 aa, Artificial Sequence
  peptide sequence
NVTNTAGTSLPSVDLLQK

SEQ ID NO: 179 - protein, 9 aa, Artificial Sequence
  peptide sequence
LGAEEAKTF

SEQ ID NO: 180 - protein, 14 aa, Artificial Sequence
  peptide sequence
ILPSDYDHAEAEAR

SEQ ID NO: 181 - protein, 14 aa, Artificial Sequence
  peptide sequence
VGSQATDFGEALVR

SEQ ID NO: 182 - protein, 12 aa, Artificial Sequence
  peptide sequence
GNSTGGFDGQAR

SEQ ID NO: 183 - protein, 20 aa, Artificial Sequence
  peptide sequence
RGQLASPSSQSAAASSLGPY

SEQ ID NO: 184 - protein, 18 aa, Artificial Sequence
  peptide sequence
RGQPGNAYDGAGQPSAAY